European Patent Application EP 4 524 256 A1, published March 19, 2025. Title: 一种双特异性探针捕获磁珠及其制备方法和应用. Applicant: 圣湘生物科技股份有限公司. The sequence listing filed with the application follows.

SEQUENCE LISTING (27 sequences)

SEQ ID NO: 1 - DNA, 40 bp, Artificial sequence
  source 1..40: mol_type = other DNA
  modified_base 26..29: mod_base = i
cggcgtttattggttttcggagttgnnnntcggcgtgtaa

SEQ ID NO: 2 - DNA, 40 bp, Artificial sequence
  source 1..40: mol_type = other DNA
  modified_base 20..23: mod_base = i
tttatcgggtattttagtcnnnnagaaggcggaagttacg

SEQ ID NO: 3 - DNA, 40 bp, Artificial sequence
  source 1..40: mol_type = other DNA
  modified_base 21..24: mod_base = i
ttagttattatgtcggatttnnnngttaacgcgtagttgg

SEQ ID NO: 4 - DNA, 36 bp, Artificial sequence
  source 1..36: mol_type = other DNA
  modified_base 22..25: mod_base = i
ttgtaatttttaagggaggagnnnnttttattggtt

SEQ ID NO: 5 - DNA, 40 bp, Artificial sequence
  source 1..40: mol_type = other DNA
  modified_base 19..22: mod_base = i
agtttatctgcaaggtgannnnttaattcctctctttcct

SEQ ID NO: 6 - DNA, 40 bp, Artificial sequence
  source 1..40: mol_type = other DNA
cggcgtttattggttttcggagttgttaatcggcgtgtaa

SEQ ID NO: 7 - DNA, 40 bp, Artificial sequence
  source 1..40: mol_type = other DNA
agtttatctgcaaggtgattccttaattcctctctttcct

SEQ ID NO: 8 - DNA, 36 bp, Artificial sequence
  source 1..36: mol_type = other DNA
ttgtaatttttaagggaggagtaggttttattggtt

SEQ ID NO: 9 - DNA, 21 bp, Artificial sequence
  source 1..21: mol_type = other DNA
cgtaggagttttggtttgtcg

SEQ ID NO: 10 - DNA, 25 bp, Artificial sequence
  source 1..25: mol_type = other DNA
acaatataactcccaaataaacccg

SEQ ID NO: 11 - DNA, 22 bp, Artificial sequence
  source 1..22: mol_type = other DNA
ttcggagttgttaatcggcgtg

SEQ ID NO: 12 - DNA, 28 bp, Artificial sequence
  source 1..28: mol_type = other DNA
tgtacaagtccacaaggaaagtaaagat

SEQ ID NO: 13 - DNA, 26 bp, Artificial sequence
  source 1..26: mol_type = other DNA
tgtttcgatgagtttatctgcaaggt

SEQ ID NO: 14 - DNA, 33 bp, Artificial sequence
  source 1..33: mol_type = other DNA
tctaactaggaccgcagaggaaagagaggaatt

SEQ ID NO: 15 - DNA, 22 bp, Artificial sequence
  source 1..22: mol_type = other DNA
gtgtgttgggtggtggttattt

SEQ ID NO: 16 - DNA, 30 bp, Artificial sequence
  source 1..30: mol_type = other DNA
ccaaaaaaaaaactacttattccaattcac

SEQ ID NO: 17 - DNA, 18 bp, Artificial sequence
  source 1..18: mol_type = other DNA
ttaagggaggagtaggtt

SEQ ID NO: 18 - DNA, 40 bp, Artificial sequence
  source 1..40: mol_type = other DNA
  modified_base 2..5: mod_base = i
cnnnntttattggttttcggagttgttaatcggcgtgtaa

SEQ ID NO: 19 - DNA, 40 bp, Artificial sequence
  source 1..40: mol_type = other DNA
  modified_base 36..39: mod_base = i
cggcgtttattggttttcggagttgttaatcggcgnnnna

SEQ ID NO: 20 - DNA, 40 bp, Artificial sequence
  source 1..40: mol_type = other DNA
tttatcgggtattttagtcgcgtagaaggcggaagttacg

SEQ ID NO: 21 - DNA, 40 bp, Artificial sequence
  source 1..40: mol_type = other DNA
  modified_base 3..6: mod_base = i
ttnnnngggtattttagtcgcgtagaaggcggaagttacg

SEQ ID NO: 22 - DNA, 40 bp, Artificial sequence
  source 1..40: mol_type = other DNA
  modified_base 35..38: mod_base = i
tttatcgggtattttagtcgcgtagaaggcggaannnncg

SEQ ID NO: 23 - DNA, 40 bp, Artificial sequence
  source 1..40: mol_type = other DNA
ttagttattatgtcggatttcgcggttaacgcgtagttgg

SEQ ID NO: 24 - DNA, 40 bp, Artificial sequence
  source 1..40: mol_type = other DNA
  modified_base 3..6: mod_base = i
ttnnnnattatgtcggatttcgcggttaacgcgtagttgg

SEQ ID NO: 25 - DNA, 40 bp, Artificial sequence
  source 1..40: mol_type = other DNA
  modified_base 35..38: mod_base = i
ttagttattatgtcggatttcgcggttaacgcgtnnnngg

SEQ ID NO: 26 - DNA, 40 bp, Artificial sequence
  source 1..40: mol_type = other DNA
ttagttattatgttggatttcgcggttaacgcgtagttgg

SEQ ID NO: 27 - DNA, 40 bp, Artificial sequence
  source 1..40: mol_type = other DNA
ttagttattatgttggatttcgcggttaatgtgtagttgg